European Patent Specification EP 4 402 471 B1, published June 25, 2025. Title: A CHEMOSELECTIVE ELECTROCATALYTIC BIOCONJUGATION REACTION AND USES THEREOF. Applicant: TRUSTEES OF BOSTON COLLEGE. The sequence listing filed with the application follows.

SEQUENCE LISTING (4 sequences)

SEQ ID NO: 1 - DNA, 8480 bp, synthetic construct
  misc_feature 1..8480: note = Description of sequence: plasmid Construct
  misc_feature 1..8480: note = Name of sequence: pCDNA3.1-C-Her2+SbfI
  misc_feature 2779..3421: note = Gene - Light chain of Trastuzumab
  misc_feature 4099..5452: note = Gene - Heavy chain of Trastuzumab
  source 1..8480: mol_type = other DNA
cgacttatcgccactggcagcagccactggtaacaggattagcagagcgaggtatgtaggcggtgctacagagttcttgaagtggtggcctaactacggctacactagaagaacagtatttggtatctgcgctctgctgaagccagttaccttcggaaaaagagttggtagctcttgatccggcaaacaaaccaccgctggtagcggtttttttgtttgcaagcagcagattacgcgcagaaaaaaaggatctcaagaagatcctttgatcttttctacggggtctgacgctcagtggaacgaaaactcacgttaagggattttggtcatgagattatcaaaaaggatcttcacctagatccttttaaattaaaaatgaagttttaaatcaatctaaagtatatatgagtaaacttggtctgacagttaccaatgcttaatcagtgaggcacctatctcagcgatctgtctatttcgttcatccatagttgcctgactccccgtcgtgtagataactacgatacgggagggcttaccatctggccccagtgctgcaatgataccgcgagacccacgctcaccggctccagatttatcagcaataaaccagccagccggaagggccgagcgcagaagtggtcctgcaactttatccgcctccatccagtctattaattgttgccgggaagctagagtaagtagttcgccagttaatagtttgcgcaacgttgttgccattgctacaggcatcgtggtgtcacgctcgtcgtttggtatggcttcattcagctccggttcccaacgatcaaggcgagttacatgatcccccatgttgtgcaaaaaagcggttagctccttcggtcctccgatcgttgtcagaagtaagttggccgcagtgttatcactcatggttatggcagcactgcataattctcttactgtcatgccatccgtaagatgcttttctgtgactggtgagtactcaaccaagtcattctgagaatagtgtatgcggcgaccgagttgctcttgcccggcgtcaatacgggataataccgcgccacatagcagaactttaaaagtgctcatcattggaaaacgttcttcggggcgaaaactctcaaggatcttaccgctgttgagatccagttcgatgtaacccactcgtgcacccaactgatcttcagcatcttttactttcaccagcgtttctgggtgagcaaaaacaggaaggcaaaatgccgcaaaaaagggaataagggcgacacggaaatgttgaatactcatactcttcctttttcaatattattgaagcatttatcagggttattgtctcatgagcggatacatatttgaatgtatttagaaaaataaacaaataggggttccgcgcacatttccccgaaaagtgccacctgacgtcgacggatcgggagatctcggccgcagcgatcgcatccatggcctccgcgaccggctgcagaacagcgggcagttcggtttcaggcaggtcttgcaacgtgacaccctgtgcacggcgggagatgcaataggtcaggctctcgctgaattccccaatgtcaagcacttccggaatcgggagcgcggccgatgcaaagtgccgataaacataacgatctttgtagaaaccatcggcgcagctatttacccgcaggacatatccacgccctcctacatcgaagctgaaagcacgagattcttcgccctccgagagctgcatcaggtcggagacgctgtcgaacttttcgatcagaaacttctcgacagacgtcgcggtgagttcaggcttaattaagtacgggcctccaaaaaagcctcctcactacttctggaatagctcagaggcagaggcggcctcggcctctgcataaataaaaaaaattagtcagccatggggcggagaatgggcggaactgggcggagttaggggcgggatgggcggagttaggggcgggactatggttgctgactaattgagatgcatgctttgcatacttctgcctgctggggagcctggggactttccacacctggttgctgactaattgagatgcatgctttgcatacttctgcccgcggagttattaatagtaatcaattacggggtcattagttcatagcccatatatggagttccgcgttacataacttacggtaaatggcccgcctggctgaccgcccaacgacccccgcccattgacgtcaataatgacgtatgttcccatagtaacgccaatagggactttccattgacgtcaatgggtggagtatttacggtaaactgcccacttggcagtacatcaagtgtatcatatgccaagtacgccccctattgacgtcaatgacggtaaatggcccgcctggcattatgcccagtacatgaccttatgggactttcctacttggcagtacatctacgtattagtcatcgctattaccatggtgatgcggttttggcagtacatcaatgggcgtggatagcggtttgactcacggggatttccaagtctccaccccattgacgtcaatgggagtttgttttggcaccaaaatcaacgggactttccaaaatgtcgtaacaactccgccccattgacgcaaatgggcggtaggcgtgtacggtgggaggtctatataagcagagctgggtacgtgaaccgtcagatcgcctggagacgccatcacactagtcaccatgagggtccccgctcagctcctggggctcctgctgctctggctcccaggtgcacgatgtgacatccagatgacccagtccccctcctccctgtctgcctccgtgggcgacagagtgaccatcacctgtcgggcctcccaggatgtgaacaccgccgtggcctggtatcagcagaagcctggcaaggcccctaagctgctgatctactccgcctccttcctgtactccggcgtgccctcccggttctccggctccagatccggcaccgacttcaccctgaccatctccagcctgcagcctgaggacttcgccacctactactgccagcagcactacaccacccctccaaccttcggccagggcaccaaggtggagatcaagcgtacggtggctgcaccatctgtcttcatcttcccgccatctgatgagcagttgaaatctggaactgcctctgttgtgtgcctgctgaataacttctatcccagagaggccaaagtacagtggaaggtggataacgccctccaatcgggtaactcccaggagagtgtcacagagcaggacagcaaggacagcacctacagcctcagcagcaccctgacgctgagcaaagcagactacgagaaacacaaagtctacgcctgcgaagtcacccatcagggcctgagctcgcccgtcacaaagagcttcaacaggggagagtgttaataacctgcaggtcactgtgccttctagttgccagccatctgttgtttgcccctcccccgtgccttccttgaccctggaaggtgccactcccactgtcctttcctaataaaatgaggaaattgcatcgcattgtctgagtaggtgtcattctattctggggggtggggtggggcaggacagcaagggggaggattgggaagacaatagcaggcatgctggggatgcggtggggtcgacatatgccaagtacgccccctattgacgtcaatgacggtaaatggcccgcctggcattatgcccagtacatgaccttatgggactttcctacttggcagtacatctacgtattagtcatcgctattaccatggtgatgcggttttggcagtacatcaatgggcgtggatagcggtttgactcacggggatttccaagcctccaccccattgacgtcaatgggagtttgttttggcaccaaaatcaacgggactttccaaaatgtcgtaacaactccgccccattgacgcaaatgggcggtaggcgtgtacggtgggaggtctatataagcagagctgggtacgtcctcacattcagtgatcagcactgaacacaggatatccaccatgggttggagcctcatcttgctcttccttgtcgctgttgctacgcgtgtccactccgaagtgcagctggtggagtctggcggaggactggtgcagccagggggcagcctgagactgtcttgcgccgcctccggcttcaacatcaaggacacctacatccactgggtccgccaggcaccaggcaagggactggaatgggtggcccggatctaccctaccaacggctacaccagatacgccgactccgtgaagggccggttcaccatctccgccgacacctccaagaacaccgcctacctgcagatgaattccctgagggccgaggacaccgccgtgtactactgctccagatggggaggcgacggcttctacgccatggactactggggccagggcaccctggtcacagtgtcctctgctagcaccaagggcccatcggtcttccccctggcaccctcctccaagagcacctctgggggcacagcggccctgggctgcctggtcaaggactacttccccgaaccggtgacggtgtcgtggaactcaggcgccctgaccagcggcgtgcacaccttcccggctgtcctacagtcctcaggactctactccctcagcagcgtggtgaccgtgccctccagcagcttgggcacccagacctacatctgcaacgtgaatcacaagcccagcaacaccaaggtggacaagaaagttgagcccaaatcttgtgacaaaactcacacatgcccaccgtgcccagcacctgaactcctggggggaccgtcagtcttcctcttccccccaaaacccaaggacaccctcatgatctcccggacccctgaggtcacatgcgtggtggtggacgtgagccacgaagaccctgaggtcaagttcaactggtacgtggacggcgtggaggtgcataatgccaagacaaagccgcgggaggagcagtacaacagcacgtaccgtgtggtcagcgtcctcaccgtcctgcaccaggactggctgaatggcaaggagtacaagtgcaaggtctccaacaaagccctcccagcccccatcgagaaaaccatctccaaagccaaagggcagccccgagaaccacaggtgtacaccctgcccccatcccgggatgagctgaccaagaaccaggtcagcctgacctgcctggtcaaaggcttctatcccagcgacatcgccgtggagtgggagagcaatgggcagccggagaacaactacaagaccacgcctcccgtgctggactccgacggctccttcttcctctacagcaagctcaccgtggacaagagcaggtggcagcaggggaacgtcttctcatgctccgtgatgcatgaggctctgcacaaccactacacgcagaagagcctctccctgtctccgggttcttaagcggccgctcgagtctagagggcccgtttaaacccgctgatcagcctcgactgtgccttctagttgccagccatctgttgtttgcccctcccccgtgccttccttgaccctggaaggtgccactcccactgtcctttcctaataaaatgaggaaattgcatcgcattgtctgagtaggtgtcattctattctggggggtggggtggggcaggacagcaagggggaggattgggaagacaatagcaggcatgctggggatgcggtgggctctatggcttctgaggcggaaagaaccagctggggctctagggggtatccccacgcgccctgtagcggcgcattaagcgcggcgggtgtggtggttacgcgcagcgtgaccgctacacttgccagcgccctagcgcccgctcctttcgctttcttcccttcctttctcgccacgttcgccggctttccccgtcaagctctaaatcgggggctccctttagggttccgatttagtgctttacggcacctcgaccccaaaaaacttgattagggtgatggttcacgtagtgggccatcgccctgatagacggtttttcgccctttgacgttggagtccacgttctttaatagtggactcttgttccaaactggaacaacactcaaccctatctcggtctattcttttgatttataagggattttgccgatttcggcctattggttaaaaaatgagctgatttaacaaaaatttaacgcgaattaattctgtggaatgtgtgtcagttagggtgtggaaagtccccaggctccccagcaggcagaagtatgcaaagcatgcatctcaattagtcagcaaccaggtgtggaaagtccccaggctccccagcaggcagaagtatgcaaagcatgcatctcaattagtcagcaaccatagtcccgcccctaactccgcccatcccgcccctaactccgcccagttccgcccattctccgccccatggctgactaattttttttatttatgcagaggccgaggccgcctctgcctctgagctattccagaagtagtgaggaggcttttttggaggcctaggcttttgcaaaaagctcccgggagcttgtatatccattttcggatctgatcaagagacaggatgaggatcgtttcgcatgattgaacaagatggattgcacgcaggttctccggccgcttgggtggagaggctattcggctatgactgggcacaacagacaatcggctgctctgatgccgccgtgttccggctgtcagcgcaggggcgcccggttctttttgtcaagaccgacctgtccggtgccctgaatgaactgcaggacgaggcagcgcggctatcgtggctggccacgacgggcgttccttgcgcagctgtgctcgacgttgtcactgaagcgggaagggactggctgctattgggcgaagtgccggggcaggatctcctgtcatctcaccttgctcctgccgagaaagtatccatcatggctgatgcaatgcggcggctgcatacgcttgatccggctacctgcccattcgaccaccaagcgaaacatcgcatcgagcgagcacgtactcggatggaagccggtcttgtcgatcaggatgatctggacgaagagcatcaggggctcgcgccagccgaactgttcgccaggctcaaggcgcgcatgcccgacggcgaggatctcgtcgtgacccatggcgatgcctgcttgccgaatatcatggtggaaaatggccgcttttctggattcatcgactgtggccggctgggtgtggcggaccgctatcaggacatagcgttggctacccgtgatattgctgaagagcttggcggcgaatgggctgaccgcttcctcgtgctttacggtatcgccgctcccgattcgcagcgcatcgccttctatcgccttcttgacgagttcttctgagcgggactctggggttcgaaatgaccgaccaagcgacgcccaacctgccatcacgagatttcgattccaccgccgccttctatgaaaggttgggcttcggaatcgttttccgggacgccggctggatgatcctccagcgcggggatctcatgctggagttcttcgcccaccccaacttgtttattgcagcttataatggttacaaataaagcaatagcatcacaaatttcacaaataaagcatttttttcactgcattctagttgtggtttgtccaaactcatcaatgtatcttatcatgtctgtataccgtcgacctctagctagagcttggcgtaatcatggtcatagctgtttcctgtgtgaaattgttatccgctcacaattccacacaacatacgagccggaagcataaagtgtaaagcctggggtgcctaatgagtgagctaactcacattaattgcgttgcgctcactgcccgctttccagtcgggaaacctgtcgtgccagctgcattaatgaatcggccaacgcgcggggagaggcggtttgcgtattgggcgctcttccgcttcctcgctcactgactcgctgcgctcggtcgttcggctgcggcgagcggtatcagctcactcaaaggcggtaatacggttatccacagaatcaggggataacgcaggaaagaacatgtgagcaaaaggccagcaaaaggccaggaaccgtaaaaaggccgcgttgctggcgtttttccataggctccgcccccctgacgagcatcacaaaaatcgacgctcaagtcagaggtggcgaaacccgacaggactataaagataccaggcgtttccccctggaagctccctcgtgcgctctcctgttccgaccctgccgcttaccggatacctgtccgcctttctcccttcgggaagcgtggcgctttctcatagctcacgctgtaggtatctcagttcggtgtaggtcgttcgctccaagctgggctgtgtgcacgaaccccccgttcagcccgaccgctgcgccttatccggtaactatcgtcttgagtccaacccggtaagaca

SEQ ID NO: 2 - DNA, 9332 bp, synthetic construct
  misc_feature 1..9332: note = Description of sequence: Plasmid construct
  misc_feature 1..9332: note = Name of sequence:pAcBac1_EcWRS1-5HTP-H14_RevU6EcW_TGA
  misc_feature 4971..5976: note = Gene - EcWRS-H14
  misc_feature 8736..8811: note = Gene - EcW tRNA UCA (TGA suppressor)
  source 1..9332: mol_type = other DNA
ttctctgtcacagaatgaaaatttttctgtcatctcttcgttattaatgtttgtaattgactgaatatcaacgcttatttgcagcctgaatggcgaatgggacgcgccctgtagcggcgcattaagcgcggcgggtgtggtggttacgcgcagcgtgaccgctacacttgccagcgccctagcgcccgctcctttcgctttcttcccttcctttctcgccacgttcgccggctttccccgtcaagctctaaatcgggggctccctttagggttccgatttagtgctttacggcacctcgaccccaaaaaacttgattagggtgatggttcacgtagtgggccatcgccctgatagacggtttttcgccctttgacgttggagtccacgttctttaatagtggactcttgttccaaactggaacaacactcaaccctatctcggtctattcttttgatttataagggattttgccgatttcggcctattggttaaaaaatgagctgatttaacaaaaatttaacgcgaattttaacaaaatattaacgtttacaatttcaggtggcacttttcggggaaatgtgcgcggaacccctatttgtttatttttctaaatacattcaaatatgtatccgctcatgagacaataaccctgataaatgcttcaataatattgaaaaaggaagagtatgagtattcaacatttccgtgtcgcccttattcccttttttgcggcattttgccttcctgtttttgctcacccagaaacgctggtgaaagtaaaagatgctgaagatcagttgggtgcacgagtgggttacatcgaactggatctcaacagcggtaagatccttgagagttttcgccccgaagaacgttttccaatgatgagcacttttaaagttctgctatgtggcgcggtattatcccgtattgacgccgggcaagagcaactcggtcgccgcatacactattctcagaatgacttggttgagtactcaccagtcacagaaaagcatcttacggatggcatgacagtaagagaattatgcagtgctgccataaccatgagtgataacactgcggccaacttacttctgacaacgatcggaggaccgaaggagctaaccgcttttttgcacaacatgggggatcatgtaactcgccttgatcgttgggaaccggagctgaatgaagccataccaaacgacgagcgtgacaccacgatgcctgtagcaatggcaacaacgttgcgcaaactattaactggcgaactacttactctagcttcccggcaacaattaatagactggatggaggcggataaagttgcaggaccacttctgcgctcggcccttccggctggctggtttattgctgataaatctggagccggtgagcgtgggtctcgcggtatcattgcagcactggggccagatggtaagccctcccgtatcgtagttatctacacgacggggagtcaggcaactatggatgaacgaaatagacagatcgctgagataggtgcctcactgattaagcattggtaactgtcagaccaagtttactcatatatactttagattgatttaaaacttcatttttaatttaaaaggatctaggtgaagatcctttttgataatctcatgaccaaaatcccttaacgtgagttttcgttccactgagcgtcagaccccgtagaaaagatcaaaggatcttcttgagatcctttttttctgcgcgtaatctgctgcttgcaaacaaaaaaaccaccgctaccagcggtggtttgtttgccggatcaagagctaccaactctttttccgaaggtaactggcttcagcagagcgcagataccaaatactgtccttctagtgtagccgtagttaggccaccacttcaagaactctgtagcaccgcctacatacctcgctctgctaatcctgttaccagtggctgctgccagtggcgataagtcgtgtcttaccgggttggactcaagacgatagttaccggataaggcgcagcggtcgggctgaacggggggttcgtgcacacagcccagcttggagcgaacgacctacaccgaactgagatacctacagcgtgagcattgagaaagcgccacgcttcccgaagggagaaaggcggacaggtatccggtaagcggcagggtcggaacaggagagcgcacgagggagcttccagggggaaacgcctggtatctttatagtcctgtcgggtttcgccacctctgacttgagcgtcgatttttgtgatgctcgtcaggggggcggagcctatggaaaaacgccagcaacgcggcctttttacggttcctggccttttgctggccttttgctcacatgttctttcctgcgttatcccctgattctgtggataaccgtattaccgcctttgagtgagctgataccgctcgccgcagccgaacgaccgagcgcagcgagtcagtgagcgaggaagcggaagagcgcctgatgcggtattttctccttacgcatctgtgcggtatttcacaccgcagaccagccgcgtaacctggcaaaatcggttacggttgagtaataaatggatgccctgcgtaagcgggtgtgggcggacaataaagtcttaaactgaacaaaatagatctaaactatgacaataaagtcttaaactagacagaatagttgtaaactgaaatcagtccagttatgctgtgaaaaagcatactggacttttgttatggctaaagcaaactcttcattttctgaagtgcaaattgcccgtcgtattaaagaggggcgtggccaagggcatggtaaagactatattcgcggcgttgtgacaatttaccgaacaactccgcggccgggaagccgatctcggcttgaacgaattgttaggtggcggtacttgggtcgatatcaaagtgcatcacttcttcccgtatgcccaactttgtatagagagccactgcgggatcgtcaccgtaatctgcttgcacgtagatcacataagcaccaagcgcgttggcctcatgcttgaggagattgatgagcgcggtggcaatgccctgcctccggtgctcgccggagactgcgagatcatagatatagatctcactacgcggctgctcaaacctgggcagaacgtaagccgcgagagcgccaacaaccgcttcttggtcgaaggcagcaagcgcgatgaatgtcttactacggagcaagttcccgaggtaatcggagtccggctgatgttgggagtaggtggctacgtctccgaactcacgaccgaaaagatcaagagcagcccgcatggatttgacttggtcagggccgagcctacatgtgcgaatgatgcccatacttgagccacctaactttgttttagggcgactgccctgctgcgtaacatcgttgctgctgcgtaacatcgttgctgctccataacatcaaacatcgacccacggcgtaacgcgcttgctgcttggatgcccgaggcatagactgtacaaaaaaacagtcataacaagccatgaaaaccgccactgcgccgttaccaccgctgcgttcggtcaaggttctggaccagttgcgtgagcgcatacgctacttgcattacagtttacgaaccgaacaggcttatgtcaactgggttcgtgccttcatccgtttccacggtgtgcgtcacccggcaaccttgggcagcagcgaagtcgaggcatttctgtcctggctggcgaacgagcgcaaggtttcggtctccacgcatcgtcaggcattggcggccttgctgttcttctacggcaaggtgctgtgcacggatctgccctggcttcaggagatcggtagacctcggccgtcgcggcgcttgccggtggtgctgaccccggatgaagtggttcgcatcctcggttttctggaaggcgagcatcgtttgttcgcccaggactctagctatagttctagtggttggctacgtacccgtagtggctatggcagggcttgcgcttaatgcgccgctacagggcgcgtggggataccccctagagccccagctggttctttccgcctcagaagccatagagcccaccgcatccccagcatgcctgctattgtcttcccaatcctcccccttgctgtcctgccccaccccaccccccagaatagaatgacacctactcagacaatgcgatgcaatttcctcattttattaggaaaggacagtgggagtggcaccttccagggtcaaggaaggcacgggggaggggcaaacaacagatggctggcaactagaaggcacagtcgaggctgatcagcgggtttaaacgggccctctagactcgagttaaagtcgacgcggggaggcggcccaaagggagatccgactcgtctgagggcgaaggcgaagacgcggaagaggccgcagagccggcagcaggccgcgggaaggaaggtccgctggattgagggccgaagggacgtagcagaaggacgtcccgcgcagaatccaggtggcaacacaggcgagcagccaaggaaaggacgatgatttccccgacaacaccacggaattgtcagtgcccaacagccgagcccctgtccagcagcgggcaaggcaggcggcgatgagttccgccgtggcaatagggagggggaaagcgaaagtcccggaaaggagctgacaggtggtggcaatgccccaaccagtgggggttgcgtcagcaaacacagtgcacaccacgccacgttgcctgacaacgggccacaactcctcataaagagacagcaaccaggatttatacaaggaggagaaaatgaaagccatacgggaagcaatagcatgatacaaaggcattaaagcagcgtatccacatagcgtaaaaggagcaacatagttaagaataccagtcaatctttcacaaattttgtaatccagaggttgattgtcgacttaacgcgttgaattcttacggcttcgccacaaaaccaatcgcttcgtacaccgcttttagcgtacgggaagcgtgcgcgctggctttttccgcgccatctttcatcacctgttgcaggaaggcttcatcgttgcggaaacggtgatagcgttcctgcaattcagtcagcataccggaaacggcatcagccacttcacctttcagatgaccatacatcttgccttcgaactgtttttccagttctgggatgctctggcccgttaccgctgaaaggatatccaacaggttggaaacgcccgctttgttctgcacatcgtagcgaactaccggcggctcgtcggagtcagtgaccgcacgtttgattttcttcactaccgatttcggatcttccagcaggccgataacgttattgcgattatcgtcagacttggacatcttcttggtcggctccagcagcgacattacgcgcgcgccagatttcggaataaacggctccggcaccttaaagatctcgccatacagcgcgttgaaacgctgggcaatatcgcggctcagttcgaggtgctgtttctggtcttcaccacaaggacccagattagtttgatacagcaggatgtccgctgccatcagcaccggatagtcaaacagaccagcgttgatgttctcggcataacgcgcagatttatctttaaactgcgtcatgcgactcagttcgccgaagtaggtatagcagttcagtgcccagcctaactgtgcatgttccggcacgtgggactgaacaaaaatggtgcttttctcaggatcgataccacaagccagatacaaggccagcgtatccagcgtcgctttacgcagcttctgtgcatcctggcgcacggtgatcgcgtgttggtcaacgatacagtaaatgcaatggtagtcatcctgcatgtttacccactgacgcagcgcacccatgtagttaccaatggtcaattcacctgagggctgtgcgccagcaaaaacgatgggcttagtcatggtggcgctagccagcttgggtctccctatagtgagtcgtattaatttcgataagccagtaagcagtgggttctctagttagccagagagctctgcttatatagacctcccaccgtacacgcctaccgcccatttgcgtcaatggggcggagttgttacgacattttggaaagtcccgttgattttggtgccaaaacaaactcccattgacgtcaatggggtggagacttggaaatccccgtgagtcaaaccgctatccacgcccattgatgtactgccaaaaccgcatcaccatggtaatagcgatgactaatacgtagatgtactgccaagtaggaaagtcccataaggtcatgtactgggcataatgccaggcgggccatttaccgtcattgacgtcaatagggggcgtacttggcatatgatacacttgatgtactgccaagtgggcagtttaccgtaaatagtccacccattgacgtcaatggaaagtccctattggcgttactatgggaacatacgtcattattgacgtcaatgggcgggggtcgttgggcggtcagccaggcgggccatttaccgtaagttatgtaacgcggaactccatatatgggctatgaactaatgaccccgtaattgattactattaataactagtcaataatcaatgtcaacgcgtatatctggcccgtacatcgcgaagcagcgcaaaacggatcctgcaggtatttgcggccgcggtccgtatactccggaatattaatagatcatggagataattaaaatgataaccatctcgcaaataaataagtattttactgttttcgtaacagttttgtaataaaaaaacctataaatattccggattattcataccgtcccaccatcgggcgcgaactcctaaaaaaccgccaccatgaagtgccttttgtacttagcctttttattcattggggtgaattgcaagttcaccatagtttttccacacaaccaaaaaggaaactggaaaaatgttccttctaattaccattattgcccgtcaagctcagatttaaattggcataatgacttaataggcacagccttacaagtcaaaatgcccaagagtcacaaggctattcaagcagacggttggatgtgtcatgcttccaaatgggtcactacttgtgatttccgctggtatggaccgaagtatataacacattccatccgatccttcactccatctgtagaacaatgcaaggaaagcattgaacaaacgaaacaaggaacttggctgaatccaggcttccctcctcaaagttgtggatatgcaactgtgacggatgccgaagcagtgattgtccaggtgactcctcaccatgtgctggttgatgaatacacaggagaatgggttgattcacagttcatcaacggaaaatgcagcaattacatatgccccactgtccataactctacaacctggcattctgactataaggtcaaagggctatgtgattctaacctcatttccatggacatcaccttcttctcagaggacggagagctatcatccctgggaaaggagggcacagggttcagaagtaactactttgcttatgaaactggaggcaaggcctgcaaaatgcaatactgcaagcattggggagtcagactcccatcaggtgtctggttcgagatggctgataaggatctctttgctgcagccagattccctgaatgcccagaagggtcaagtatctctgctccatctcagacctcagtggatgtaagtctaattcaggacgttgagaggatcttggattattccctctgccaagaaacctggagcaaaatcagagcgggtcttccaatctctccagtggatctcagctatcttgctcctaaaaacccaggaaccggtcctgctttcaccataatcaatggtaccctaaaatactttgagaccagatacatcagagtcgatattgctgctccaatcctctcaagaatggtcggaatgatcagtggaactaccacagaaagggaactgtgggatgactgggcaccatatgaagacgtggaaattggacccaatggagttctgaggaccagttcaggatataagtttcctttatacatgattggacatggtatgttggactccgatcttcatcttagctcaaaggctcaggtgttcgaacatcctcacattcaagacgctgcttcgcaacttcctgatgatgagagtttattttttggtgatactgggctatccaaaaatccaatcgagcttgtagaaggttggttcagtagttggaaaagctctattgcctcttttttctttatcatagggttaatcattggactattcttggttctccgagttggtatccatctttgcattaaattaaagcacaccaagaaaagacagatttatacagacatagagatgaaccgacttggaaagtgataaggccaggccggccaagcttgtcgagaagtactagaggatcataatcagccataccacatttgtagaggttttacttgctttaaaaaacctcccacacctccccctgaacctgaaacataaaatgaatgcaattgttgttgttaacttgtttattgcagcttataatggttacaaataaagcaatagcatcacaaatttcacaaataaagcatttttttcactgcattctagttgtggtttgtccaaactcatcaatgtatcttatcatgtctggatctgatcactgcttgagcctagcaaaaaatggcaggggcggagagactcgaactcccaacacccggttttgaagaccggtgctctaccaattgaactacgcccctggtgtttcgtcctttccacaagatatataaagccaagaaatcgaaatactttcaagttacggtaagcatatgatagtccattttaaaacataattttaaaactgcaaactacccaagaaattattactttctacgtcacgtattttgtactaatatctttgtgtttacagtcaaattaattctaattatctctctaacagccttgtatcgtatatgcaaatatgaaggaatcatgggaaataggccctcttcctgcccgacctaggagatccgaaccagataagtgaaatctagttccaaactattttgtcatttttaattttcgtattagcttacgacgctacacccagttcccatctattttgtcactcttccctaaataatccttaaaaactccatttccacccctcccagttcccaactattttgtccgcccacagcggggcatttttcttcctgttatgtttttaatcaaacatcctgccaactccatgtgacaaaccgtcatcttcggctacttt

SEQ ID NO: 3 - DNA, 5986 bp, synthetic construct
  misc_feature 1..5986: note = Description of sequence: Plasmid Construct
  misc_feature 1..5986: note = Name of sequence: pET22b-T5-5F7 sequence
  misc_feature 5304..5559: note = Gene - 5F7 (AntiHer2 nanobody)
  source 1..5986: mol_type = other DNA
tggcgaatgggacgcgccctgtagcggcgcattaagcgcggcgggtgtggtggttacgcgcagcgtgaccgctacacttgccagcgccctagcgcccgctcctttcgctttcttcccttcctttctcgccacgttcgccggctttccccgtcaagctctaaatcgggggctccctttagggttccgatttagtgctttacggcacctcgaccccaaaaaacttgattagggtgatggttcacgtagtgggccatcgccctgatagacggtttttcgccctttgacgttggagtccacgttctttaatagtggactcttgttccaaactggaacaacactcaaccctatctcggtctattcttttgatttataagggattttgccgatttcggcctattggttaaaaaatgagctgatttaacaaaaatttaacgcgaattttaacaaaatattaacgtttacaatttcaggtggcacttttcggggaaatgtgcgcggaacccctatttgtttatttttctaaatacattcaaatatgtatccgctcatgagacaataaccctgataaatgcttcaataatattgaaaaaggaagagtatgagtattcaacatttccgtgtcgcccttattcccttttttgcggcattttgccttcctgtttttgctcacccagaaacgctggtgaaagtaaaagatgctgaagatcagttgggtgcacgagtgggttacatcgaactggatctcaacagcggtaagatccttgagagttttcgccccgaagaacgttttccaatgatgagcacttttaaagttctgctatgtggcgcggtattatcccgtattgacgccgggcaagagcaactcggtcgccgcatacactattctcagaatgacttggttgagtactcaccagtcacagaaaagcatcttacggatggcatgacagtaagagaattatgcagtgctgccataaccatgagtgataacactgcggccaacttacttctgacaacgatcggaggaccgaaggagctaaccgcttttttgcacaacatgggggatcatgtaactcgccttgatcgttgggaaccggagctgaatgaagccataccaaacgacgagcgtgacaccacgatgcctgcagcaatggcaacaacgttgcgcaaactattaactggcgaactacttactctagcttcccggcaacaattaatagactggatggaggcggataaagttgcaggaccacttctgcgctcggcccttccggctggctggtttattgctgataaatctggagccggtgagcgtgggtctcgcggtatcattgcagcactggggccagatggtaagccctcccgtatcgtagttatctacacgacggggagtcaggcaactatggatgaacgaaatagacagatcgctgagataggtgcctcactgattaagcattggtaactgtcagaccaagtttactcatatatactttagattgatttaaaacttcatttttaatttaaaaggatctaggtgaagatcctttttgataatctcatgaccaaaatcccttaacgtgagttttcgttccactgagcgtcagaccccgtagaaaagatcaaaggatcttcttgagatcctttttttctgcgcgtaatctgctgcttgcaaacaaaaaaaccaccgctaccagcggtggtttgtttgccggatcaagagctaccaactctttttccgaaggtaactggcttcagcagagcgcagataccaaatactgtccttctagtgtagccgtagttaggccaccacttcaagaactctgtagcaccgcctacatacctcgctctgctaatcctgttaccagtggctgctgccagtggcgataagtcgtgtcttaccgggttggactcaagacgatagttaccggataaggcgcagcggtcgggctgaacggggggttcgtgcacacagcccagcttggagcgaacgacctacaccgaactgagatacctacagcgtgagctatgagaaagcgccacgcttcccgaagggagaaaggcggacaggtatccggtaagcggcagggtcggaacaggagagcgcacgagggagcttccagggggaaacgcctggtatctttatagtcctgtcgggtttcgccacctctgacttgagcgtcgatttttgtgatgctcgtcaggggggcggagcctatggaaaaacgccagcaacgcggcctttttacggttcctggccttttgctggccttttgctcacatgttctttcctgcgttatcccctgattctgtggataaccgtattaccgcctttgagtgagctgataccgctcgccgcagccgaacgaccgagcgcagcgagtcagtgagcgaggaagcggaagagcgcctgatgcggtattttctccttacgcatctgtgcggtatttcacaccgcatatatggtgcactctcagtacaatctgctctgatgccgcatagttaagccagtatacactccgctatcgctacgtgactgggtcatggctgcgccccgacacccgccaacacccgctgacgcgccctgacgggcttgtctgctcccggcatccgcttacagacaagctgtgaccgtctccgggagctgcatgtgtcagaggttttcaccgtcatcaccgaaacgcgcgaggcagctgcggtaaagctcatcagcgtggtcgtgaagcgattcacagatgtctgcctgttcatccgcgtccagctcgttgagtttctccagaagcgttaatgtctggcttctgataaagcgggccatgttaagggcggttttttcctgtttggtcactgatgcctccgtgtaagggggatttctgttcatgggggtaatgataccgatgaaacgagagaggatgctcacgatacgggttactgatgatgaacatgcccggttactggaacgttgtgagggtaaacaactggcggtatggatgcggcgggaccagagaaaaatcactcagggtcaatgccagcgcttcgttaatacagatgtaggtgttccacagggtagccagcagcatcctgcgatgcagatccggaacataatggtgcagggcgctgacttccgcgtttccagactttacgaaacacggaaaccgaagaccattcatgttgttgctcaggtcgcagacgttttgcagcagcagtcgcttcacgttcgctcgcgtatcggtgattcattctgctaaccagtaaggcaaccccgccagcctagccgggtcctcaacgacaggagcacgatcatgcgcacccgtggggccgccatgccggcgataatggcctgcttctcgccgaaacgtttggtggcgggaccagtgacgaaggcttgagcgagggcgtgcaagattccgaataccgcaagcgacaggccgatcatcgtcgcgctccagcgaaagcggtcctcgccgaaaatgacccagagcgctgccggcacctgtcctacgagttgcatgataaagaagacagtcataagtgcggcgacgatagtcatgccccgcgcccaccggaaggagctgactgggttgaaggctctcaagggcatcggtcgagatcccggtgcctaatgagtgagctaacttacattaattgcgttgcgctcactgcccgctttccagtcgggaaacctgtcgtgccagctgcattaatgaatcggccaacgcgcggggagaggcggtttgcgtattgggcgccagggtggtttttcttttcaccagtgagacgggcaacagctgattgcccttcaccgcctggccctgagagagttgcagcaagcggtccacgctggtttgccccagcaggcgaaaatcctgtttgatggtggttaacggcgggatataacatgagctgtcttcggtatcgtcgtatcccactaccgagatatccgcaccaacgcgcagcccggactcggtaatggcgcgcattgcgcccagcgccatctgatcgttggcaaccagcatcgcagtgggaacgatgccctcattcagcatttgcatggtttgttgaaaaccggacatggcactccagtcgccttcccgttccgctatcggctgaatttgattgcgagtgagatatttatgccagccagccagacgcagacgcgccgagacagaacttaatgggcccgctaacagcgcgatttgctggtgacccaatgcgaccagatgctccacgcccagtcgcgtaccgtcttcatgggagaaaataatactgttgatgggtgtctggtcagagacatcaagaaataacgccggaacattagtgcaggcagcttccacagcaatggcatcctggtcatccagcggatagttaatgatcagcccactgacgcgttgcgcgagaagattgtgcaccgccgctttacaggcttcgacgccgcttcgttctaccatcgacaccaccacgctggcacccagttgatcggcgcgagatttaatcgccgcgacaatttgcgacggcgcgtgcagggccagactggaggtggcaacgccaatcagcaacgactgtttgcccgccagttgttgtgccacgcggttgggaatgtaattcagctccgccatcgccgcttccactttttcccgcgttttcgcagaaacgtggctggcctggttcaccacgcgggaaacggtctgataagagacaccggcatactctgcgacatcgtataacgttactggtttcacattcaccaccctgaattgactctcttccgggcgctatcatgccataccgcgaaaggttttgcgccattcgatggtgtccgggatctcgacgctctcccttatgcgactcctgcattaggaagcagcccagtagtaggttgaggccgttgagcaccgccgccgcaaggaatggtgcatgcaaggagatggcgcccaacagtcccccggccacggggcctgccaccatacccacgccgaaacaagcgctcatgagcccgaagtggcgagcccgatcttccccatcggtgatgtcggcgatataggcgccagcaaccgcacctgtggcgccggtgatgccggccacgatgcgtccggcgtagaggatcgagatctcgatcccgcgaaattaatacgactcactataggggaattgtgagcggataacaattcccctctagagtttgacagcattatcatcgatctcgagaaatcataaaaaatttatttgctttgtgagcggataacaattataatagattcaattgtgagcggataacaatttcacacagaattcattaaagaggagaaattacatatggaagtgcagctggtggaaagcggcggcggccttgtgcaggcgggcggcagcctgcgcctgagctgcgcggcgagcggcattacctttagcattaacacgatgggctggtatcgccaggcgccgggcaaacagcgcgaactggtggcgctgattagcagcattggcgatacctattatgcggatagcgtgaaaggccgcttttggattagccgcgataacgcgaaaaacaccgtgtatctgcaaatgaacagcctgaaaccggaagataccgcggtgtattattgcaaacgctttcgcaccgcggcgcagggcaccgattattggggccagggcacccaagtgaccgtgagcagccatcaccaccaccatcactaaaagcttaattagctgagcttggactcctgttgatagatccagtaatgacctcagaactccatctggatttgttcagaacgctcggttgccgccgggcgttttttattggtgagaatccaagctagcttggcggcggccgcactcgagcaccaccaccaccaccactgagatccggctgctaacaaagcccgaaaggaagctgagttggctgctgccaccgctgagcaataactagcataaccccttggggcctctaaacgggtcttgaggggttttttgctgaaaggaggaactatatccggat

SEQ ID NO: 4 - DNA, 6106 bp, synthetic construct
  misc_feature 1..6106: note = Description of sequence: Plasmid Construct
  misc_feature 1..6106: note = Name of sequence: pET22b-Myoglobin-K99>TAG
  misc_feature 3302..3394: note = Gene - Myoglobin
  source 1..6106: mol_type = other DNA
agatacctacagcgtgagctatgagaaagcgccacgcttcccgaagggagaaaggcggacaggtatccggtaagcggcagggtcggaacaggagagcgcacgagggagcttccagggggaaacgcctggtatctttatagtcctgtcgggtttcgccacctctgacttgagcgtcgatttttgtgatgctcgtcaggggggcggagcctatggaaaaacgccagcaacgcggcctttttacggttcctggccttttgctggccttttgctcacatgttctttcctgcgttatcccctgattctgtggataaccgtattaccgcctttgagtgagctgataccgctcgccgcagccgaacgaccgagcgcagcgagtcagtgagcgaggaagcggaagagcgcctgatgcggtattttctccttacgcatctgtgcggtatttcacaccgcatatatggtgcactctcagtacaatctgctctgatgccgcatagttaagccagtatacactccgctatcgctacgtgactgggtcatggctgcgccccgacacccgccaacacccgctgacgcgccctgacgggcttgtctgctcccggcatccgcttacagacaagctgtgaccgtctccgggagctgcatgtgtcagaggttttcaccgtcatcaccgaaacgcgcgaggcagctgcggtaaagctcatcagcgtggtcgtgaagcgattcacagatgtctgcctgttcatccgcgtccagctcgttgagtttctccagaagcgttaatgtctggcttctgataaagcgggccatgttaagggcggttttttcctgtttggtcactgatgcctccgtgtaagggggatttctgttcatgggggtaatgataccgatgaaacgagagaggatgctcacgatacgggttactgatgatgaacatgcccggttactggaacgttgtgagggtaaacaactggcggtatggatgcggcgggaccagagaaaaatcactcagggtcaatgccagcgcttcgttaatacagatgtaggtgttccacagggtagccagcagcatcctgcgatgcagatccggaacataatggtgcagggcgctgacttccgcgtttccagactttacgaaacacggaaaccgaagaccattcatgttgttgctcaggtcgcagacgttttgcagcagcagtcgcttcacgttcgctcgcgtatcggtgattcattctgctaaccagtaaggcaaccccgccagcctagccgggtcctcaacgacaggagcacgatcatgcgcacccgtggggccgccatgccggcgataatggcctgcttctcgccgaaacgtttggtggcgggaccagtgacgaaggcttgagcgagggcgtgcaagattccgaataccgcaagcgacaggccgatcatcgtcgcgctccagcgaaagcggtcctcgccgaaaatgacccagagcgctgccggcacctgtcctacgagttgcatgataaagaagacagtcataagtgcggcgacgatagtcatgccccgcgcccaccggaaggagctgactgggttgaaggctctcaagggcatcggtcgagatcccggtgcctaatgagtgagctaacttacattaattgcgttgcgctcactgcccgctttccagtcgggaaacctgtcgtgccagctgcattaatgaatcggccaacgcgcggggagaggcggtttgcgtattgggcgccagggtggtttttcttttcaccagtgagacgggcaacagctgattgcccttcaccgcctggccctgagagagttgcagcaagcggtccacgctggtttgccccagcaggcgaaaatcctgtttgatggtggttaacggcgggatataacatgagctgtcttcggtatcgtcgtatcccactaccgagatatccgcaccaacgcgcagcccggactcggtaatggcgcgcattgcgcccagcgccatctgatcgttggcaaccagcatcgcagtgggaacgatgccctcattcagcatttgcatggtttgttgaaaaccggacatggcactccagtcgccttcccgttccgctatcggctgaatttgattgcgagtgagatatttatgccagccagccagacgcagacgcgccgagacagaacttaatgggcccgctaacagcgcgatttgctggtgacccaatgcgaccagatgctccacgcccagtcgcgtaccgtcttcatgggagaaaataatactgttgatgggtgtctggtcagagacatcaagaaataacgccggaacattagtgcaggcagcttccacagcaatggcatcctggtcatccagcggatagttaatgatcagcccactgacgcgttgcgcgagaagattgtgcaccgccgctttacaggcttcgacgccgcttcgttctaccatcgacaccaccacgctggcacccagttgatcggcgcgagatttaatcgccgcgacaatttgcgacggcgcgtgcagggccagactggaggtggcaacgccaatcagcaacgactgtttgcccgccagttgttgtgccacgcggttgggaatgtaattcagctccgccatcgccgcttccactttttcccgcgttttcgcagaaacgtggctggcctggttcaccacgcgggaaacggtctgataagagacaccggcatactctgcgacatcgtataacgttactggtttcacattcaccaccctgaattgactctcttccgggcgctatcatgccataccgcgaaaggttttgcgccattcgatggtgtccgggatctcgacgctctcccttatgcgactcctgcattaggaagcagcccagtagtaggttgaggccgttgagcaccgccgccgcaaggaatggtgcatgcaaggagatggcgcccaacagtcccccggccacggggcctgccaccatacccacgccgaaacaagcgctcatgagcccgaagtggcgagcccgatcttccccatcggtgatgtcggcgatataggcgccagcaaccgcacctgtggcgccggtgatgccggccacgatgcgtccggcgtagaggatcgagatctcgatcccgcgaaattaatacgactcactataggggaattgtgagcggataacaattcccctctagagtttgacagcattatcatcgatctcgagaaatcataaaaaatttatttgctttgtgagcggataacaattataatagattcaattgtgagcggataacaatttcacacagaattcattaaagaggagaaattacatatggttctgtctgaaggtgaatggcagctggttctgcatgtttgggctaaagttgaagctgacgtcgctggtcatggtcaggacatcttgattcgactgttcaaatctcatccggaaactctggaaaaattcgatcgtttcaaacatctgaaaactgaagctgaaatgaaagcttctgaagatctgaaaaaacatggtgttaccgtgttaactgccctaggtgctatccttaagaaaaaagggcatcatgaagctgagctcaaaccgcttgcacaatcgcatgctactaaacataagatcccgatcaaatacctggaattcatctctgaagcgatcatccatgttctgcattctagacatccaggtgacttcggtgctgacgctcagggtgctatgaacaaagctctcgagctgttccgtaaagatatcgctgctaagtacaaagaactgggttagcagggtggctcgggacatcatcaccatcaccattaaggtctcaagcttaattagctgagcttggactcctgttgatagatccagtaatgacctcagaactccatctggatttgttcagaacgctcggttgccgccgggcgttttttattggtgagaatccaagctagcttggcggcggccgcactcgagcaccaccaccaccaccactgagatccggctgctaacaaagcccgaaaggaagctgagttggctgctgccaccgctgagcaataactagcataaccccttggggcctctaaacgggtcttgaggggttttttgctgaaaggaggaactatatccggattggcgaatgggacgcgccctgtagcggcgcattaagcgcggcgggtgtggtggttacgcgcagcgtgaccgctacacttgccagcgccctagcgcccgctcctttcgctttcttcccttcctttctcgccacgttcgccggctttccccgtcaagctctaaatcgggggctccctttagggttccgatttagtgctttacggcacctcgaccccaaaaaacttgattagggtgatggttcacgtagtgggccatcgccctgatagacggtttttcgccctttgacgttggagtccacgttctttaatagtggactcttgttccaaactggaacaacactcaaccctatctcggtctattcttttgatttataagggattttgccgatttcggcctattggttaaaaaatgagctgatttaacaaaaatttaacgcgaattttaacaaaatattaacgtttacaatttcaggtggcacttttcggggaaatgtgcgcggaacccctatttgtttatttttctaaatacattcaaatatgtatccgctcatgagacaataaccctgataaatgcttcaataatattgaaaaaggaagagtatgagtattcaacatttccgtgtcgcccttattcccttttttgcggcattttgccttcctgtttttgctcacccagaaacgctggtgaaagtaaaagatgctgaagatcagttgggtgcacgagtgggttacatcgaactggatctcaacagcggtaagatccttgagagttttcgccccgaagaacgttttccaatgatgagcacttttaaagttctgctatgtggcgcggtattatcccgtattgacgccgggcaagagcaactcggtcgccgcatacactattctcagaatgacttggttgagtactcaccagtcacagaaaagcatcttacggatggcatgacagtaagagaattatgcagtgctgccataaccatgagtgataacactgcggccaacttacttctgacaacgatcggaggaccgaaggagctaaccgcttttttgcacaacatgggggatcatgtaactcgccttgatcgttgggaaccggagctgaatgaagccataccaaacgacgagcgtgacaccacgatgcctgcagcaatggcaacaacgttgcgcaaactattaactggcgaactacttactctagcttcccggcaacaattaatagactggatggaggcggataaagttgcaggaccacttctgcgctcggcccttccggctggctggtttattgctgataaatctggagccggtgagcgtgggtctcgcggtatcattgcagcactggggccagatggtaagccctcccgtatcgtagttatctacacgacggggagtcaggcaactatggatgaacgaaatagacagatcgctgagataggtgcctcactgattaagcattggtaactgtcagaccaagtttactcatatatactttagattgatttaaaacttcatttttaatttaaaaggatctaggtgaagatcctttttgataatctcatgaccaaaatcccttaacgtgagttttcgttccactgagcgtcagaccccgtagaaaagatcaaaggatcttcttgagatcctttttttctgcgcgtaatctgctgcttgcaaacaaaaaaaccaccgctaccagcggtggtttgtttgccggatcaagagctaccaactctttttccgaaggtaactggcttcagcagagcgcagataccaaatactgtccttctagtgtagccgtagttaggccaccacttcaagaactctgtagcaccgcctacatacctcgctctgctaatcctgttaccagtggctgctgccagtggcgataagtcgtgtcttaccgggttggactcaagacgatagttaccggataaggcgcagcggtcgggctgaacggggggttcgtgcacacagcccagcttggagcgaacgacctacaccgaactg